European Patent Specification EP 3 658 669 B1, published June 5, 2024. Title: Mutated cellobiose dehydrogenase with modified substrate. Applicant: Directsens GmbH. The sequence listing filed with the application follows.

SEQUENCE LISTING (17 sequences)

SEQ ID NO: 1 - protein, 831 aa, Chaetomium atrobrunneum
MRPSSRFVGALAAAASFLPSALAQNNAAVTFTDPDTGIVFNSWGLANGAPQTQGGFTFGVALPSDALTTDATEFIGYLECASADNQGWCGVSMGGPMTNSLLITAWPHEDNVYTSLRFATGYAMPDVYSGDATITQISSSINATHFKLIFRCQNCLQWTHDGASGGASTSAGVLVLGWVQAFPSPGNPTCPDQITLEQHNNGMGIWGAVMDSNVANPSYTEWAAQATKTVEAECDGPSETDIVGVPVPTGTTFDYIVVGGGAGGIPTADKLSEAGKSVLLIEKGIASTAEHGGTLGPEWLEGNDLTRFDVPGLCNQIWVDSKGIACEDTDQMAGCVLGGGTAVNAGLWFKPYSLDWDYLFPSGWKYRDIQAAIGRVFSRIPGTDAPSTDGKRYYQQGFDVLAGGLSAGGWNKVTANSSPDKKNRTFSNAPFMFSGGERGGPLATYLTSAKKRSNFNLWLNTSVKRVIREGGHVTGVEVEPFRTGGYQGIVNVTAVSGRVVLSAGTFGSAKILLRGGIGPADQLEVVKASKIDGPTMISNASWIPLPVGYNLDDHLNTDTVITHPDVAFYDFYEAWNTPIEADKNSYLSSRTGILAQAAPNIGPMMWEEIKGADGIVRQLQWTARVEGSFDTPNGQAMTISQYLGRGATSRGRMTITPSLTTVVSDVPYLKDPNDKEAVIQGIVNLQNALKNVAGLTWTYPNSSITPREYVDNMVVSPSNRRANHWMGTAKIGTDDGRLAGGSAVVDLNTKVYGTDNLFVVDASIFPGTPTTNPSAYIVTAAEHASQRILGLAAPKPVGKWGQCGGRQWTGSFQCVSGTKCEVVNEWYSQCL

SEQ ID NO: 2 - protein, 845 aa, Hypoxylon haematostroma
MGRLGSLAKLLLAVGLNVQQCFGQNGPPTPYTDSETGITFATWSVPDRAEGGNGLAPWGGLTFGVALPENALTTDATELIGYLKCGSNGTTTDAWCGLSFGGPMTNSLLLMAWPHEDEILTSFRFASGYTRPDLYTGDAKLTQISSTIDKDHFTLIFRCQNCLAWNQDGASGSASTSAGSLILGWASALRAPTNAGCPAEINFNFHNNGQMIWGATLDESAANPSYSEWAAKATATVTGDCGGATPTTTTTTTTSVPTATGIPVPTGTYDYIVVGAGAGGIPLADKLSEAGKSVLLIEKGPPSSGRWGGTLKPEWLKDTNLTRFDVPGLCNEIWVNSAGVACTDTDQMAGCVLGGGTAVNAGLWWKPYNLDWDYNFPRGWKSRDMAAATRRVFSRIPGTDNPSMDGKRYLQQGFEILAGGLKAAGWTEVTANDAPNKKNHTYSHSPFMFSGGERGGPMGTYLVSASRRKNFHLWTGTAVKRVVRTGGHITGLEVEPFVNGGYTGVVNVTSITGRVVLSAGAFGSAKILLRSGIGPEDQLEIVKSSTDGPTMISDSSWITLPVGYNLEDHTNTDTVVTHPDVVFYDFYEAGHPNVTDKDLYLNSRAGILAQAAPNIGPMFWEEIKGKDGVVRQLQWTARVEGSAGTPNGYAMTMSQYLGRGAKSRGRMTITKALTTVVSTVPYLQDKNDVEAVIQGIKNLQAALSNVKNLTWTYPPSNTTVEDFVNNMLVSYTNRRSNHWIGTNKLGTDDGRSRGGSAVVDLNTKVYGTDNLFVVDAGIFPGHITTNPTSYIVIAAERASERILDLPPARAQPRFAQCGGRTWTGSFQCAAPYTCQYRNERYSQCR

SEQ ID NO: 3 - protein, 787 aa, Corynascus thermophilus
MKLLSRVGATALAATLSLKQCAAQMTEGTYTHEATGITFKTWTPSDGSTFTFGLALPGDALTNDATEYIGLLRCQITDPSSPGYCGISHGQSGQMTQALLLVAWASEDVVYTSFRYATGYTLPELYTGDAKLTQIASSVSGDSFEVLFRCENCFSWDQNGATGSVSTSNGALVLGYAASKSGLTGATCPDTAEFGFHNNGFGQWGAVLEGATSDSYEEWAQLATITPPTTCDGNGPGDKVCVPAPEDTYDYIVVGAGAGGITVADKLSEAGHKVLLIEKGPPSTGLWNGTMKPEWLEGTDLTRFDVPGLCNQIWVDSAGIACTDTDQMAGCVLGGGTAVNAGLWWKPHPADWDDNFPHGWKSSDLADATERVFSRIPGTWHPSQDGKLYRQEGFEVISQGLANAGWREVDANQEPSEKNRTYSHSVFMFSGGERGGPLATYLASAAQRSNFNLWVNTSVRRAIRTGPRVSGVELECLADGGFNGTVNLKEGGGVIFSAGAFGSAKLLLRSGIGPEDQLEIVASSKDGETFISKNDWIKLPVGHNLIDHLNTDLIITHPDVVFYDFYAAWDNPITEDKEAYLNSRSGILAQAAPNIGPLMWEEVTPSDGITRQFQWTCRVEGDSSKTNSTHAMTLSQYLGRGVVSRGRMGITSGLTTTVAEHPYLHNDGDLEAVIQGIQNVVDALSQVPDLEWVLPPPNTTVEEYVNSLIVSPANRRANHWMGTAKMGLDDGRSGGSAVVDLNTKVYGTDNLFVVDASIFPGMSTGNPSAMIVIVAEQAAQRILSLRY

SEQ ID NO: 4 - protein, 829 aa, Neurospora crassa
MRTTSAFLSGLAAVASLLSPAFAQTAPKTFTHPDTGIVFNTWSASDSQTKGGFTVGMALPSNALTTDATEFIGYLECSSAKNGANSGWCGVSLRGAMTNNLLITAWPSDGEVYTNLMFATGYAMPKNYAGDAKITQIASSVNATHFTLVFRCQNCLSWDQDGVTGGISTSNKGAQLGWVQAFPSPGNPTCPTQITLSQHDNGMGQWGAAFDSNIANPSYTAWAAKATKTVTGTCSGPVTTSIAATPVPTGVSFDYIVVGGGAGGIPVADKLSESGKSVLLIEKGFASTGEHGGTLKPEWLNNTSLTRFDVPGLCNQIWKDSDGIACSDTDQMAGCVLGGGTAINAGLWYKPYTKDWDYLFPSGWKGSDIAGATSRALSRIPGTTTPSQDGKRYLQQGFEVLANGLKASGWKEVDSLKDSEQKNRTFSHTSYMYINGERGGPLATYLVSAKKRSNFKLWLNTAVKRVIREGGHITGVEVEAFRNGGYSGIIPVTNTTGRVVLSAGTFGSAKILLRSGIGPKDQLEVVKASADGPTMVSNSSWIDLPVGHNLVDHTNTDTVIQHNNVTFYDFYKAWDNPNTTDMNLYLNGRSGIFAQAAPNIGPLFWEEITGADGIVRQLHWTARVEGSFETPDGYAMTMSQYLGRGATSRGRMTLSPTLNTVVSDLPYLKDPNDKAAVVQGIVNLQKALANVKGLTWAYPSANQTAADFVDKQPVTYQSRRSNHWMGTNKMGTDDGRSGGTAVVDTNTRVYGTDNLYVVDASIFPGVPTTNPTAYIVVAAEHAAAKILAQPANEAVPKWGWCGGPTYTGSQTCQAPYKCEKQNDWYWQCV

SEQ ID NO: 5 - protein, 828 aa, Myriococcum thermophilum [sequence omitted]

SEQ ID NO: 6 - protein, 829 aa, Stachybotrys bisbyi
MLFKLSNWLLALALFVGNVVAQLVGPTPYTDPDTGIVFQSWVNPAGTLKFGYTYPANAATVAATEFIGFLECQGAGWCSVSLGGSMLNKPLVVAYPSGDEVLASLKWATGYANPEPYGGNHKLSQISSSVTSAGFRVVYRCEGCLAWNYQGIEGGSPTNGASMPIGWAYSASSVLNGDCVDNTVLIQHDTFGNYGFVPDESSLRTEYNDWTELPTRVVRGDCGGSTTTSSVPSSTAPPQGTGIPVPTGASYDYIVVGSGAGGIPIADKLTEAGKKVLLIEKGPPSSGRYDGKLKPTWLEGTNLTRFDVPGLCNQIWVDSAGIACRDTDQMAGCVLGGGTAVNAGLWWKPNPIDWDYNFPSGWKSSEMIGATNRVFSRIGGTTVPSQDGKTYYQQGFNVLSSGLKAAGWTSVSLNNAPAQKNRTYGAGPFMFSGGERGGPLATYLATAKKRGNFDLWTNTQVKRVIRQGGHVTGVEVENYNGDGYKGTVKVTPVSGRVVLSAGTFGSAKLLLRSGIGPKDQLAIVKNSTDGPTMASERDWINLPVGYNLEDHTNTDIVISHPDVVHYDFYEAWTAPIESDKTAYLGKRSGILAQAAPNIGPLFFDEVRGADNIVRSIQYTARVEGNSVVPNGKAMVISQYLGRGAVSRGRMTISQGLNTIVSTAPYLSNVNDLEAVIKSLENIANSLTSKVKNLKIEWPASGTSIRDHVTNMPLDPATRRANHWIGTNKIGTKDGRLTGGDSVVDLNTKVYGTDNLFVVDASIFPGMVTTNPSAYIVIAAEHAASKILSLPTAKAAAKYEQCGGLEYNGNFQCASGLTCTWLNDYYWQCT

SEQ ID NO: 7 - protein, 771 aa, Athelia rolfsii
MLSRLVLNLLAITVIGVFGQSSSSYTDNGINFQGITDPTYGVTYGAVFPPASVDSDEFIGEIAAPVAAKWIGLSLGGAMINNLLIVAWPNNNEIVFSSRYTTGYVLPTIYSGPKITTISSSVNSTHWKWIYRCQNCTTWSGGSLAANGSAVWAWAYSSAAVDTPSSPSSSFDEHTDFGFFGEITSNAHVSQSVYEQYLTGTGVTSTSSSTSTTTSTSTTTSTSSAPTVSATPYDYIIVGAGPAGIIAADRLSEAGKKVLLLERGGPSTKETGGTYTAPWAASSGLTKFDIPGVFESLFTDSNSFWWCKDITVFAGCLTGGGTAINGALYWYPTDLDFSTANGWPSSWTAHQKYTDLVSSRLPSSDHPSTDGKRYLEQSAAVVAQLLNGQGYRNKTINNAPNAKDHVYGYSAFDFLNGKRAGPVATYLQTAKTRNNFHFKNYVLVSNVVRNGSTITGVKTNDTSLGPNGVIPLTKNGRVILSAGSLSSPRILFQSGIGPTDMLTLVQNNPTASANLPSQSQWIHLPVGYNVADAPSINFVFTHPSIDAYDNWANVWTNPRSTDAEQYLKNQSGVLAASSPKLNFWRAYGGSDGRTRWMQGTVRPGAASINTTYNYNASQIFTITTYVSTGITSRGRIGVTSSLNVLPLVNPWLVDPVDEKVLTQSLEDLVSNMKSVPGLTMIMPDNTTSIADYVKNYDRASMNSNHWVGSNKIASNATEGVVDEHTKVFRTDNLFIVDASIIPSLPMGNPQGALMSAAEQAVAKILALAGGP

SEQ ID NO: 8 - protein, 774 aa, Gelatoporia subvermispora
MFGRFLLALLPLVGSVLSQSGSSYTDPDNGFVFNGITDPVYGVTYGVVFPEPSSSGTYPDEFIGEIVAPLTAEWIGVSFGGAMLDCLLLVAWPNQNSIVASTRYATDYVQPTEYDGPVLTTLPSSYVNSTHWKYVYRCQNCTTWQGGGISLGGTGVLAWAYSNVGVDDPSDPESNFLEHTDFGFFGENFGQTENANYNNYVNGNPGTPTSTPPTTSPTGPTTTSPASPPTASATPYDYIIVGAGAGGIIAADRLSQNNKKVLLLERGGPSTGETGGTYVADWAEGTNLTKFDIPGLFESMFDDPDPWYWCSDVTFYAGCLLGGGTSVNGALYWYPTDTDFSTARGWPSSWSNHQAYTNAMTQRLPSTDHPSTDGERYLEQSAQVAMQLLNAQGYYQATINDSPDSKDHVYGYSAFDFINGKRGGVVATYLQTANQRSNFVYKDYTLVSSVVRNGSQILGVQTNNTAIGPNGFIPLNPNGRVILSAGSFGTPRILFQSGIGPTDMLQTVQQNAAVAANMPSESDWINLPVGMNVSDNPSINLVFTHPSIDAYDNWADVWTDPRPADAAQYLASQSGVFAGASPKLNFWRDYEGSDGIQRSAQGTVRPGAASVNTTLPYNASQIFTITVYLSSGITSRGRIGVTAGLNAVALENPWLTDPVDKVVLIQALEDVISTLPSVPDLTMITPDSGMTLEEYVDLYDPSTMCSNHWVGSAKMGTSSDTAVVDENAKVFNTDNLFVIDASIVPSLPVGNPHGTVMSAAEQAVANILALSGGP

SEQ ID NO: 9 - protein, 773 aa, Phanerochaete chrysosporium
MLGRSLLALLPFVGLAFSQSASQFTDPTTGFQFTGITDPVHDVTYGFVFPPLATSGAQSTEFIGEVVAPIASKWIGIALGGAMNNDLLLVAWANGNQIVSSTRWATGYVQPTAYTGTATLTTLPETTINSTHWKWVFRCQGCTEWNNGGGIDVTSQGVLAWAFSNVAVDDPSDPQSTFSEHTDFGFFGIDYSTAHSANYQNYLNGDSGNPTTTSTKPTSTSSSVTTGPTVSATPYDYIIVGAGPGGIIAADRLSEAGKKVLLLERGGPSTKQTGGTYVAPWATSSGLTKFDIPGLFESLFTDSNPFWWCKDITVFAGCLVGGGTSVNGALYWYPNDGDFSSSVGWPSSWTNHAPYTSKLSSRLPSTDHPSTDGQRYLEQSFNVVSQLLKGQGYNQATINDNPNYKDHVFGYSAFDFLNGKRAGPVATYLQTALARPNFTFKTNVMVSNVVRNGSQILGVQTNDPTLGPNGFIPVTPKGRVILSAGAFGTSRILFQSGIGPTDMIQTVQSNPTAAAALPPQNQWINLPVGMNAQDNPSINLVFTHPSIDAYENWADVWSNPRPADAAQYLANQSGVFAGASPKLNFWRAYSGSDGFTRYAQGTVRPGAASVNSSLPYNASQIFTITVYLSTGIQSRGRIGIDAALRGTVLTPPWLVNPVDKTVLLQALHDVVSNIGSIPGLTMITPDVTQTLEEYVDAYDPATMNSNHWVSSTTIGSSPQSAVVDSNVKVFGTNNLFIVDAGIIPHLPTGNPQGTLMSAAEQAAAKILALAGGP

SEQ ID NO: 10 - protein, 768 aa, Trametes versicolor
MKFKSLLLSLLPLVGSVYSQVAAPYVDSGNGFVFDGVTDPVHSVTYGIVLPQASTSTEFIGEFVAPNEAQWIGLALGGAMIGNLLLVAWPDGNKIVSSPRYATGYTLPAAYAGPTITQLPSSSVNSTHWKFVFRCQNCTAWNGGSIDPSGTGVFAWAFSNVAVDDPSDPNSSFAEHTDFGFFGINFPDAQSSNYQNYLAGNAGTPPPTSVPSGPSSTTTTTGPTATATPFDYIVVGAGPGGLVTADRLSEAGKKVLLLERGGPSTAETGGTYDATWAKSANLTKFDVPGLFETLFTDTNPFWWCKDTNFFAGCLLGGGTSVNGALYWYPNSRDFSTASGWPSSWGNHQPFTDKLKQRLPSTDHPSADGQRYLEQSATVVQQLLSGQGYSQITINDNPDSKDHVFGFSAFDFLNGQRAGPVATYFETALARKNFVYKDNVLVTQVIRNGSTILGVRTNDNTLGPDGIVPLNPNGRVILSGGSFGTPRILFQSGIGPTDMLQTVQSNAQAAANLPPQSEWINLPVGQSVSDNPSINLVFTHPSIDAYDNWADVWSNPRPADAQQYLQSRSGVLAGASPKLNFWRAYGGSDGITRYAQGTVRPGAASVNTSVAYNASEIFTITLYLSNGIQSRGRIGVDAALNAKALVNPWLTNSVDKTVLLQALHDVTSTMKNVPGLTMITPDNTMTLEQYVAAYDPATMCSNHWVGAAKMGTSSSTAVVDENAKVFNTDNLFIVDASIIPSLPIGNPQGVLMSAAEQAVSRILALAGGP

SEQ ID NO: 11 - DNA, 23 bp, Artificial sequence
  primer
caacaccgaaaccgtcatccagc

SEQ ID NO: 12 - DNA, 22 bp, Artificial sequence
  primer
gatgacggtttcggtgttggtg

SEQ ID NO: 13 - DNA, 23 bp, Artificial Sequence
  primer
caacaccgttaccgtcatccagc

SEQ ID NO: 14 - DNA, 22 bp, Artificial Sequence
  primer
gatgacggtaacggtgttggtg

SEQ ID NO: 15 - DNA, 33 bp, Artificial Sequence
  primer
gccatgaccatgaaccagtaccttggccgtggc

SEQ ID NO: 16 - DNA, 21 bp, Artificial Sequence
  primer
catggtcatggcgtagccgtc

SEQ ID NO: 17 - protein, 785 aa, Humicola insolens
MKFLGRIGATALAASLYLTSGAAQATGDAYTDSETGIKFQTWSPDPQFTFGLALPPDALEKDATEYIGLLRCTRADPSDPGYCGLSHGQVGQMTQSLLLVAWAYENQVYTSFRYATGYTLPGLYTGNAKLTQLSVNITDTSFELIYRCENCFSWEHEGSTGSSSTSQGYLVLGRASARRGVVGPTCPDTATFGFHDNGFGQWGVGLENAVSEQYSEWASLPGLTVETTCEGSGPGEAQCVPAPEETYDYIVVGAGAGGIPVADKLSEAGHKVLLIEKGPPSTGRWQGTMKPEWLEGTDLTRFDVPGLCNQIWVDSAGIACTDTDQMAGCVLGGGTAVNAGLWWKPIDLDWDENFPEGWHSQDLAAATERVFERIPGTWHPSMDGKLYRDEGYKVLSSGLAESGWKEVVANEVPNEKNRTFAHTHFMFAGGERNGPLATYLVSADARENFSLWTNTAVRRAVRTGGKVTGVELECLTDGGYSGIVKLNEGGGVIFSAGAFGSAKLLFRSGIGPEDQLRVVASSKDGEDFIDEKDWIKLPVGYNLIDHLNTDLILTHPDVVFYDFYEAWTTPIEADKQLYLEQRSGILAQAAPNIGPMMWEQVTPSDGITRQFQWTARVEGDSRFTNSSHAMTLSQYLGRGVVSRGRATITQGLVTTVAEHPYLHNAGDKEAVIQGIKNLIESLNVIPNITWVLPPPGSTVEEYVDSLLVSASARRSNHWMGTAKLGTDDGRYGGTSVVDLDTKVYGTDNLFVVDASIFPGMSTGNPSAMIVIAAEQAAERILKLRK